European Patent Application EP 4 023 677 A9, published January 4, 2023. Title: Anti-TFPI monoclonal antibodies. Applicant: SUZHOU ALPHAMAB CO., LTD. The sequence listing filed with the application follows.

SEQUENCE LISTING (28 sequences)

SEQ ID NO: 1 - DNA, 27 bp, Artificial Sequence
  primer KF-1-EcoRV
  misc_feature (10)..(10): k is G or T
  misc_feature (13)..(13): m is A or C
  misc_feature (15)..(15): s is C or G
  misc_feature (22)..(22): w is A or T
ggtgatatcktgmtsacccaawctcca

SEQ ID NO: 2 - DNA, 32 bp, Artificial Sequence
  primer KR-BamHI
gggaagatggatccagttggtgcagcatcagc

SEQ ID NO: 3 - DNA, 22 bp, Artificial Sequence
  primer GF-2-PstI
aggtsmaactgcagsagtcwgg

SEQ ID NO: 4 - DNA, 38 bp, Artificial Sequence
  primer GR-HindIII
ccaggggccagtggatagacaagcttgggtgtcgtttt

SEQ ID NO: 5 - DNA, 363 bp, Artificial Sequence
  7G6VH
caggttcagctgcagcagtctggagctgaactggcgaggcctggggcttcagtgaagctgtcctgcaaggcttctggctacagcttcacaagttatggtataagttgggtgaagcagagaactggacagggccttgagtggatcggagagatttatcctagaagtactaatacttactacaatgagaagttcatgggcaaggccacactgactgcagacaaatcctccagcacagcgttcatggagctccgcagcctgacatctgaggactctgcggtctatttctgtgcaagagaatccttctatggtgactatggggctatggacttctggggtcagggagcctcagtcaccgtctcctca

SEQ ID NO: 6 - protein, 121 aa, Artificial Sequence
  7G6VH
QVQLQQSGAELARPGASVKLSCKASGYSFTSYGISWVKQRTGQGLEWIGEIYPRSTNTYYNEKFMGKATLTADKSSSTAFMELRSLTSEDSAVYFCARESFYGDYGAMDFWGQGASVTVSS

SEQ ID NO: 7 - protein, 5 aa, Artificial Sequence
  7G6 VH CDR1 KABAT
SYGIS

SEQ ID NO: 8 - protein, 17 aa, Artificial Sequence
  7G6 VH CDR2 KABAT
EIYPRSTNTYYNEKFMG

SEQ ID NO: 9 - protein, 12 aa, Artificial Sequence
  7G6 VH CDR3 KABAT
ESFYGDYGAMDF

SEQ ID NO: 10 - DNA, 290 bp, Artificial Sequence
  7G6VL
gatatcgtgctgacccaatctccactcactttgtcggttaccattggacaaccagcctccatcttttgcaagtcaagtcagagcctcttagaaagtgatggaaagacatatttgaattggttgttgcagaggccaggccagtctccaaagcgccttatctatctggtgtctaaactggactctggagtccctgacaggttcactggcagtggatcagggacagatttcacactgaagatcagcagagtggaggctgaggatttgggagtttattattgctgccaaggtac

SEQ ID NO: 11 - protein, 112 aa, Artificial Sequence
  7G6VL
DIVLTQSPLTLSVTIGQPASIFCKSSQSLLESDGKTYLNWLLQRPGQSPKRLIYLVSKLDSGVPDRFTGSGSGTDFTLKISRVEAEDLGVYYCCQGTHFPRTFGGGTKLEIK

SEQ ID NO: 12 - protein, 16 aa, Artificial Sequence
  7G6 VL CDR1 KABAT
KSSQSLLESDGKTYLN

SEQ ID NO: 13 - protein, 7 aa, Artificial Sequence
  7G6 VL CDR2 KABAT
LVSKLDS

SEQ ID NO: 14 - protein, 8 aa, Artificial Sequence
  7G6 VL CDR3 KABAT
QGTHFPRT

SEQ ID NO: 15 - protein, 121 aa, Artificial Sequence
  h7G6VH-v1
QVQLVQSGAEVKKPGASVKVSCKASGYTFTSYGISWVRQAPGQGLEWMGEIYPRSTNTYYNEKFMGRVTMTRDKSSSTAYMELSSLRSEDTAVYYCARESFYGDYGAMDFWGQGTLVTVSS

SEQ ID NO: 16 - protein, 121 aa, Artificial Sequence
  hu7G6VH-v2
QVQLVQSGAEVKKPGASVKVSCKASGYSFTSYGISWVKQAPGQGLEWIGEIYPRSTNTYYNEKFMGKATLTADKSSSTAYMELSSLRSEDTAVYYCARESFYGDYGAMDFWGQGTLVTVSS

SEQ ID NO: 17 - protein, 112 aa, Artificial Sequence
  h7G6VL-v1
DIVMTQSPLSLPVTPGEPASISCKSSQSLLESDGKTYLNWYLQKPGQSPQLLIYLVSKLDSGVPDRFSGSGSGTDFTLKISRVEAEDVGVYYCWQGTHFPRTFGQGTKVEIK

SEQ ID NO: 18 - protein, 112 aa, Artificial Sequence
  h7G6VL-v2
DIVLTQSPLSLPVTPGEPASIFCKSSQSLLESDGKTYLNWLLQKPGQSPQRLIYLVSKLDSGVPDRFSGSGSGTDFTLKISRVEAEDVGVYYCSQGTHFPRTFGQGTKVEIK

SEQ ID NO: 19 - protein, 112 aa, Artificial Sequence
  7G6VL-v3
DIVMTQSPLSLPVTPGEPASISCKSSQSLLESDGKTYLNWYLQKPGQSPQLLIYLVSKLDSGVPDRFSGSGSGTDFTLKISRVEAEDVGVYYCSQGTHFPRTFGQGTKVEIK

SEQ ID NO: 20 - protein, 327 aa, Artificial Sequence
  mutant human IgG4-Fc region
ASTKGPSVFPLAPCSRSTSESTAALGCLVKDYFPEPVTVSWNSGALTSGVHTFPAVLQSSGLYSLSSVVTVPSSSLGTKTYTCNVDHKPSNTKVDKRVESKYGPPCPPCPAPEFLGGPSVFLFPPKPKDTLMISRTPEVTCVVVDVSQEDPEVQFNWYVDGVEVHNAKTKPREEQFNSTYRVVSVLTVLHQDWLNGKEYKCKVSNKGLPSSIEKTISKAKGQPREPQVYTLPPSQEEMTKNQVSLTCLVKGFYPSDIAVEWESNGQPENNYKTTPPVLDSDGSFFLYSRLTVDKSRWQEGNVFSCSVMHEALHNHYTQKSLSLSLGK

SEQ ID NO: 21 - protein, 448 aa, Artificial Sequence
  h7G6 antibody heavy chain 1
QVQLVQSGAEVKKPGASVKVSCKASGYTFTSYGISWVRQAPGQGLEWMGEIYPRSTNTYYNEKFMGRVTMTRDKSSSTAYMELSSLRSEDTAVYYCARESFYGDYGAMDFWGQGTLVTVSSASTKGPSVFPLAPCSRSTSESTAALGCLVKDYFPEPVTVSWNSGALTSGVHTFPAVLQSSGLYSLSSVVTVPSSSLGTKTYTCNVDHKPSNTKVDKRVESKYGPPCPPCPAPEFLGGPSVFLFPPKPKDTLMISRTPEVTCVVVDVSQEDPEVQFNWYVDGVEVHNAKTKPREEQFNSTYRVVSVLTVLHQDWLNGKEYKCKVSNKGLPSSIEKTISKAKGQPREPQVYTLPPSQEEMTKNQVSLTCLVKGFYPSDIAVEWESNGQPENNYKTTPPVLDSDGSFFLYSRLTVDKSRWQEGNVFSCSVMHEALHNHYTQKSLSLSLGK

SEQ ID NO: 22 - protein, 448 aa, Artificial Sequence
  h7G6 antibody heavy chain 2
QVQLVQSGAEVKKPGASVKVSCKASGYSFTSYGISWVKQAPGQGLEWIGEIYPRSTNTYYNEKFMGKATLTADKSSSTAYMELSSLRSEDTAVYYCARESFYGDYGAMDFWGQGTLVTVSSASTKGPSVFPLAPCSRSTSESTAALGCLVKDYFPEPVTVSWNSGALTSGVHTFPAVLQSSGLYSLSSVVTVPSSSLGTKTYTCNVDHKPSNTKVDKRVESKYGPPCPPCPAPEFLGGPSVFLFPPKPKDTLMISRTPEVTCVVVDVSQEDPEVQFNWYVDGVEVHNAKTKPREEQFNSTYRVVSVLTVLHQDWLNGKEYKCKVSNKGLPSSIEKTISKAKGQPREPQVYTLPPSQEEMTKNQVSLTCLVKGFYPSDIAVEWESNGQPENNYKTTPPVLDSDGSFFLYSRLTVDKSRWQEGNVFSCSVMHEALHNHYTQKSLSLSLGK

SEQ ID NO: 23 - protein, 106 aa, Artificial Sequence
  ÈËIg kappa constant region
TVAAPSVFIFPPSDEQLKSGTASVVCLLNNFYPREAKVQWKVDNALQSGNSQESVTEQDSKDSTYSLSSTLTLSKADYEKHKVYACEVTHQGLSSPVTKSFNRGEC

SEQ ID NO: 24 - protein, 219 aa, Artificial Sequence
  h7G6 light chain 1
DIVMTQSPLSLPVTPGEPASISCKSSQSLLESDGKTYLNWYLQKPGQSPQLLIYLVSKLDSGVPDRFSGSGSGTDFTLKISRVEAEDVGVYYCWQGTHFPRTFGQGTKVEIKRTVAAPSVFIFPPSDEQLKSGTASVVCLLNNFYPREAKVQWKVDNALQSGNSQESVTEQDSKDSTYSLSSTLTLSKADYEKHKVYACEVTHQGLSSPVTKSFNRGEC

SEQ ID NO: 25 - protein, 219 aa, Artificial Sequence
  h7G6 light chain 2
DIVLTQSPLSLPVTPGEPASIFCKSSQSLLESDGKTYLNWLLQKPGQSPQRLIYLVSKLDSGVPDRFSGSGSGTDFTLKISRVEAEDVGVYYCSQGTHFPRTFGQGTKVEIKRTVAAPSVFIFPPSDEQLKSGTASVVCLLNNFYPREAKVQWKVDNALQSGNSQESVTEQDSKDSTYSLSSTLTLSKADYEKHKVYACEVTHQGLSSPVTKSFNRGEC

SEQ ID NO: 26 - protein, 219 aa, Artificial Sequence
  h7G6 light chain 3
DIVMTQSPLSLPVTPGEPASISCKSSQSLLESDGKTYLNWYLQKPGQSPQLLIYLVSKLDSGVPDRFSGSGSGTDFTLKISRVEAEDVGVYYCSQGTHFPRTFGQGTKVEIKRTVAAPSVFIFPPSDEQLKSGTASVVCLLNNFYPREAKVQWKVDNALQSGNSQESVTEQDSKDSTYSLSSTLTLSKADYEKHKVYACEVTHQGLSSPVTKSFNRGEC

SEQ ID NO: 27 - protein, 160 aa, Artificial Sequence
  hTFPI-K1K2
DSEEDEEHTIITDTELPPLKLMHSFCAFKADDGPCKAIMKRFFFNIFTRQCEEFIYGGCEGNQNRFESLEECKKMCTRDNANRIIKTTLQQEKPDFCFLEEDPGICRGYITRYFYNNQTKQCERFKYGGCLGNMNNFETLEECKNICEDGPNGFQVDNYG

SEQ ID NO: 28 - protein, 304 aa, Homo sapiens
MIYTMKKVHALWASVCLLLNLAPAPLNADSEEDEEHTIITDTELPPLKLMHSFCAFKADDGPCKAIMKRFFFNIFTRQCEEFIYGGCEGNQNRFESLEECKKMCTRDNANRIIKTTLQQEKPDFCFLEEDPGICRGYITRYFYNNQTKQCERFKYGGCLGNMNNFETLEECKNICEDGPNGFQVDNYGTQLNAVNNSLTPQSTKVPSLFEFHGPSWCLTPADRGLCRANENRFYYNSVIGKCRPFKYSGCGGNENNFTSKQECLRACKKGFIQRISKGGLIKTKRKRKKQRVKIAYEEIFVKNM